European Patent Application EP 4 714 972 A1, published March 25, 2026. Title: 特异性结合CD38的抗体及其制法和应用. Applicant: 亘喜生物科技（上海）有限公司. The sequence listing filed with the application follows.

SEQUENCE LISTING (20 sequences)

SEQ ID NO: 1 - protein, 124 aa, synthetic construct
QVQLVESGGGEVQPGGSLRLSCTASGFRLDYYAIGWFRRAPGKEREGIACIDITGIHTNYGDSVMGRFTISRDDRAVYLQMNNLEAGDTAIYYCAPARFSACSALDVKLSFTSWGQGTQVTVSS

SEQ ID NO: 2 - protein, 126 aa, synthetic construct
QVQLVESGGGLVQPGGSLTLSCRASGFTLDYYAIGWFRQAPGKEREAIACIDITGFHTNYGDSVSGRFTISRDNAGTTVYLQMNSLEAEDTGIYYCAPARYAACSALDVKLSFTSWGQGTQVTVSS

SEQ ID NO: 3 - protein, 116 aa, synthetic construct
QVQLVESGGGLVQAGGSLRLACTASGNIFASQVMNWYRQAPGSPRELVATITPGGRTTYADSAKGRFTVATDNAKATAYLQLTSLTPEDTGVYYCHVRLFPATDYWGQGTQVTVSS

SEQ ID NO: 4 - protein, 126 aa, synthetic construct
QVQLVESGGGLVQPGGSLRLSCTASGFRLDYYAIGWFRQAPGKEREAISCIDITGMHTNYGDSVMGRFTISRDDAKRTVYLQMNSLEAEDTGIYYCAPAQYAACSALGVKVSFTSWGQGTQVTVSP

SEQ ID NO: 5 - protein, 126 aa, synthetic construct
QVQLVESGGGLVQPGGSLRLSCTASGFRLDYYAIGWFRQAPGKEREAIACIDITGFHTNYGDSVSGRFTISRDNAGTTVYLQMNSLEAEDTGIYYCAPARYAACSALDVKLSFTSWGQGTQVTVSS

SEQ ID NO: 6 - protein, 107 aa, synthetic construct [sequence omitted]

SEQ ID NO: 7 - protein, 120 aa, synthetic construct
EVQLLESGGGLVQPGGSLRLSCAVSGFTFNSFAMSWVRQAPGKGLEWVSAISGSGGGTYYADSVKGRFTISRDNSKNTLYLQMNSLRAEDTAVYFCAKDKILWFGEPVFDYWGQGTLVTV

SEQ ID NO: 8 - protein, 15 aa, synthetic construct
GGGGSGGGGSGGGGS

SEQ ID NO: 9 - protein, 242 aa, synthetic construct
EIVLTQSPATLSLSPGERATLSCRASQSVSSYLAWYQQKPGQAPRLLIYDASNRATGIPARFSGSGSGTDFTLTISSLEPEDFAVYYCQQRSNWPPTFGQGTKVEIKGGGGSGGGGSGGGGSEVQLLESGGGLVQPGGSLRLSCAVSGFTFNSFAMSWVRQAPGKGLEWVSAISGSGGGTYYADSVKGRFTISRDNSKNTLYLQMNSLRAEDTAVYFCAKDKILWFGEPVFDYWGQGTLVTV

SEQ ID NO: 10 - protein, 21 aa, synthetic construct
MALPVTALLLPLALLLHAARP

SEQ ID NO: 11 - protein, 8 aa, synthetic construct
DYKDDDDK

SEQ ID NO: 12 - protein, 69 aa, synthetic construct
TTTPAPRPPTPAPTIASQPLSLRPEACRPAAGGAVHTRGLDFACDIYIWAPLAGTCGVLLLSLVITLYC

SEQ ID NO: 13 - protein, 42 aa, synthetic construct
KRGRKKLLYIFKQPFMRPVQTTQEEDGCSCRFPEEEEGGCEL

SEQ ID NO: 14 - protein, 112 aa, synthetic construct
RVKFSRSADAPAYKQGQNQLYNELNLGRREEYDVLDKRRGRDPEMGGKPRRKNPQEGLYNELQKDKMAEAYSEIGMKGERRRGKGHDGLYQGLSTATKDTYDALHMQALPPR

SEQ ID NO: 15 - protein, 379 aa, synthetic construct
MALPVTALLLPLALLLHAARPQVQLVESGGGEVQPGGSLRLSCTASGFRLDYYAIGWFRRAPGKEREGIACIDITGIHTNYGDSVMGRFTISRDDRAVYLQMNNLEAGDTAIYYCAPARFSACSALDVKLSFTSWGQGTQVTVSSAAADYKDDDDKTTTPAPRPPTPAPTIASQPLSLRPEACRPAAGGAVHTRGLDFACDIYIWAPLAGTCGVLLLSLVITLYCKRGRKKLLYIFKQPFMRPVQTTQEEDGCSCRFPEEEEGGCELRVKFSRSADAPAYKQGQNQLYNELNLGRREEYDVLDKRRGRDPEMGGKPRRKNPQEGLYNELQKDKMAEAYSEIGMKGERRRGKGHDGLYQGLSTATKDTYDALHMQALPPR

SEQ ID NO: 16 - protein, 381 aa, synthetic construct
MALPVTALLLPLALLLHAARPQVQLVESGGGLVQPGGSLTLSCRASGFTLDYYAIGWFRQAPGKEREAIACIDITGFHTNYGDSVSGRFTISRDNAGTTVYLQMNSLEAEDTGIYYCAPARYAACSALDVKLSFTSWGQGTQVTVSSAAADYKDDDDKTTTPAPRPPTPAPTIASQPLSLRPEACRPAAGGAVHTRGLDFACDIYIWAPLAGTCGVLLLSLVITLYCKRGRKKLLYIFKQPFMRPVQTTQEEDGCSCRFPEEEEGGCELRVKFSRSADAPAYKQGQNQLYNELNLGRREEYDVLDKRRGRDPEMGGKPRRKNPQEGLYNELQKDKMAEAYSEIGMKGERRRGKGHDGLYQGLSTATKDTYDALHMQALPPR

SEQ ID NO: 17 - protein, 371 aa, synthetic construct
MALPVTALLLPLALLLHAARPQVQLVESGGGLVQAGGSLRLACTASGNIFASQVMNWYRQAPGSPRELVATITPGGRTTYADSAKGRFTVATDNAKATAYLQLTSLTPEDTGVYYCHVRLFPATDYWGQGTQVTVSSAAADYKDDDDKTTTPAPRPPTPAPTIASQPLSLRPEACRPAAGGAVHTRGLDFACDIYIWAPLAGTCGVLLLSLVITLYCKRGRKKLLYIFKQPFMRPVQTTQEEDGCSCRFPEEEEGGCELRVKFSRSADAPAYKQGQNQLYNELNLGRREEYDVLDKRRGRDPEMGGKPRRKNPQEGLYNELQKDKMAEAYSEIGMKGERRRGKGHDGLYQGLSTATKDTYDALHMQALPPR

SEQ ID NO: 18 - protein, 381 aa, synthetic construct
MALPVTALLLPLALLLHAARPQVQLVESGGGLVQPGGSLRLSCTASGFRLDYYAIGWFRQAPGKEREAISCIDITGMHTNYGDSVMGRFTISRDDAKRTVYLQMNSLEAEDTGIYYCAPAQYAACSALGVKVSFTSWGQGTQVTVSPAAADYKDDDDKTTTPAPRPPTPAPTIASQPLSLRPEACRPAAGGAVHTRGLDFACDIYIWAPLAGTCGVLLLSLVITLYCKRGRKKLLYIFKQPFMRPVQTTQEEDGCSCRFPEEEEGGCELRVKFSRSADAPAYKQGQNQLYNELNLGRREEYDVLDKRRGRDPEMGGKPRRKNPQEGLYNELQKDKMAEAYSEIGMKGERRRGKGHDGLYQGLSTATKDTYDALHMQALPPR

SEQ ID NO: 19 - protein, 381 aa, synthetic construct
MALPVTALLLPLALLLHAARPQVQLVESGGGLVQPGGSLRLSCTASGFRLDYYAIGWFRQAPGKEREAIACIDITGFHTNYGDSVSGRFTISRDNAGTTVYLQMNSLEAEDTGIYYCAPARYAACSALDVKLSFTSWGQGTQVTVSSAAADYKDDDDKTTTPAPRPPTPAPTIASQPLSLRPEACRPAAGGAVHTRGLDFACDIYIWAPLAGTCGVLLLSLVITLYCKRGRKKLLYIFKQPFMRPVQTTQEEDGCSCRFPEEEEGGCELRVKFSRSADAPAYKQGQNQLYNELNLGRREEYDVLDKRRGRDPEMGGKPRRKNPQEGLYNELQKDKMAEAYSEIGMKGERRRGKGHDGLYQGLSTATKDTYDALHMQALPPR

SEQ ID NO: 20 - protein, 497 aa, synthetic construct
MALPVTALLLPLALLLHAARPEIVLTQSPATLSLSPGERATLSCRASQSVSSYLAWYQQKPGQAPRLLIYDASNRATGIPARFSGSGSGTDFTLTISSLEPEDFAVYYCQQRSNWPPTFGQGTKVEIKGGGGSGGGGSGGGGSEVQLLESGGGLVQPGGSLRLSCAVSGFTFNSFAMSWVRQAPGKGLEWVSAISGSGGGTYYADSVKGRFTISRDNSKNTLYLQMNSLRAEDTAVYFCAKDKILWFGEPVFDYWGQGTLVTVAAADYKDDDDKTTTPAPRPPTPAPTIASQPLSLRPEACRPAAGGAVHTRGLDFACDIYIWAPLAGTCGVLLLSLVITLYCKRGRKKLLYIFKQPFMRPVQTTQEEDGCSCRFPEEEEGGCELRVKFSRSADAPAYKQGQNQLYNELNLGRREEYDVLDKRRGRDPEMGGKPRRKNPQEGLYNELQKDKMAEAYSEIGMKGERRRGKGHDGLYQGLSTATKDTYDALHMQALPPR